European Patent Specification EP 3 042 912 B1, published February 25, 2026. Title: Immunoglobulin-binding protein. Applicant: Protenova CO., LTD. The sequence listing filed with the application follows.

SEQUENCE LISTING (12 sequences)

SEQ ID NO: 1 - protein, 58 aa, Staphylococcus aureus
  Protein A mutated immunoglobulin-binding domain(C-domain + G29A)
ADNKFNKEQQNAFYEILHLPNLTEEQRNAFIQSLKDDPSVSKEILAEAKKLNDAQAPK

SEQ ID NO: 2 - protein, 58 aa, Artificial Sequence
  modified immunoglobulin-binding protein(PN-95f)
ADNAFNTEQQNAFYEILHLPNLTEEQRNAFIQSLRDDPSVSREILAEARRLNDAQAPR

SEQ ID NO: 3 - protein, 58 aa, Artificial Sequence
  modified immunoglobulin-binding protein(PN-26f)
ADNAFNTEQQNAFYEILHLPNLTEEQRNAFIQSLRDDPSKSKKILKEAKKLNKAQAPK

SEQ ID NO: 4 - DNA, 38 bp, Artificial Sequence
  Description of Artificial Sequence: primer
cgaattctcatatggcacagcacgacgaagctgataac

SEQ ID NO: 5 - DNA, 31 bp, Artificial Sequence
  Description of Artificial Sequence: primer
ctggatccgccggggcctgtgcgtcgttcag

SEQ ID NO: 6 - DNA, 33 bp, Artificial Sequence
  Description of Artificial Sequence: primer
cgaattcaggccccgcgcgcagataacgcattt

SEQ ID NO: 7 - DNA, 32 bp, Artificial Sequence
  Description of Artificial Sequence: primer
ctggatccttatttcggtgcctgggctttgtt

SEQ ID NO: 8 - protein, 58 aa, Staphylococcus aureus
  Protein A mutated immunoglobulin-binding domain(PN-23f)
ADNKFNKEQQNAFYEILHLPNLTEEQRNAFIQSLRDDPSVSKEILAEAKKLNDAQAPK

SEQ ID NO: 9 - protein, 58 aa, Artificial Sequence
  modified immunoglobulin-binding protein(PN-28f)
ADNAFNTEQQNAFYEILHLPNLTEEQRNAFIQSLRDDPSKSKKILKEAKKLNKKQKPK

SEQ ID NO: 10 - protein, 58 aa, Staphylococcus aureus
  Protein A mutated immunoglobulin-binding domain(PN-61f)
ADNAFNTEQQNAFYEILHLPNLTEEQRNAFIQSLRDDPSVSKEILAEAKKLNDAQAPK

SEQ ID NO: 11 - protein, 58 aa, Artificial Sequence
  modified immunoglobulin-binding protein(PN-83f)
ADNKFNKEQQNAFYEILHLPNLTEEQRNAFIQSLRDDPSKSKKILKEAKKLNKAQAPK

SEQ ID NO: 12 - protein, 58 aa, Staphylococcus aureus
  Protein A mutated immunoglobulin-binding domain(PN-87f)
ADNAFNKEQQNAFYEILHLPNLTEEQRNAFIQSLRDDPSVSKEILAEAKKLNDAQAPK